European Patent Application EP 4 473 967 A1, published December 11, 2024. Title: メラノコルチン１受容体アゴニストの新規用途. Applicant: 田辺三菱製薬株式会社. Application JP. The sequence listing filed with the application follows.

SEQUENCE LISTING (6 sequences)

SEQ ID NO: 1 - DNA, 23 bp, synthetic construct
  misc_feature 1..23: note = GAPDH-F
  source 1..23: mol_type = other DNA
acccactcctccaccacctttga

SEQ ID NO: 2 - DNA, 22 bp, synthetic construct
  misc_feature 1..22: note = GAPDH-R
  source 1..22: mol_type = other DNA
ctgttgctgtagccaaattcgt

SEQ ID NO: 3 - DNA, 20 bp, synthetic construct
  misc_feature 1..20: note = ACTA2-F
  source 1..20: mol_type = other DNA
tgtatgtggctatccaggcg

SEQ ID NO: 4 - DNA, 20 bp, synthetic construct
  misc_feature 1..20: note = ACTA2-R
  source 1..20: mol_type = other DNA
agagtccagcacgatgccag

SEQ ID NO: 5 - DNA, 20 bp, synthetic construct
  misc_feature 1..20: note = COL1A1-F
  source 1..20: mol_type = other DNA
gctccgaccctgccgatgtg

SEQ ID NO: 6 - DNA, 22 bp, synthetic construct
  misc_feature 1..22: note = COL1A1-R
  source 1..22: mol_type = other DNA
catcaggcgcaggaaggtcagc